European Patent Specification EP 4 021 929 B1, published April 26, 2023. Title: hAM15-52 analogues with improved amylin receptor (hAMY3R) potency. Applicant: Gubra. The sequence listing filed with the application follows.

SEQUENCE LISTING (392 sequences)

SEQ ID NO: 1 - protein, 38 aa, Artificial Sequence
  Designed polypeptide
GCRFGTCTVQKLAHQIYQFTDKDKDNVAPRSKISPQGY

SEQ ID NO: 2 - protein, 37 aa, Artificial Sequence [sequence omitted]

SEQ ID NO: 3 - protein, 38 aa, Artificial Sequence
  Designed polypeptide
  misc_feature (38)..(38): X = Hyp (L-hydroxyproline)
KCNFATCTVQRLAHQIYQFTDKDKDNVAPRTKVGSNGX

SEQ ID NO: 4 - protein, 38 aa, Artificial Sequence
  Designed polypeptide
  misc_feature (38)..(38): X = Hyp (L-hydroxyproline)
KCNTATCTVDRLAHQIYQFTDKDKDNVAPPTNVGSNGX

SEQ ID NO: 5 - protein, 38 aa, Artificial Sequence
  Designed polypeptide
  misc_feature (38)..(38): X = Hyp (L-hydroxyproline)
KCNTATCTVQRLADQIYQFTDKDKDNVAPPTNVGSNGX

SEQ ID NO: 6 - protein, 38 aa, Artificial Sequence
  Designed polypeptide
  misc_feature (38)..(38): X = Hyp (L-hydroxyproline)
KCNTATCTVQRLAEQIYQFTDKDKDNVAPPTNVGSKGX

SEQ ID NO: 7 - protein, 38 aa, Artificial Sequence
  Designed polypeptide
  misc_feature (38)..(38): X = Hyp (L-hydroxyproline)
KCNTATCTVQRLAAQIYQFTDKDKDNVAPPTNVGSNGX

SEQ ID NO: 8 - protein, 38 aa, Artificial Sequence
  Designed polypeptide
  misc_feature (38)..(38): X = Hyp (L-hydroxyproline)
KCNTSTCTVARLADQITQFSNKDKAQVSPPTEVGPNSX

SEQ ID NO: 9 - protein, 38 aa, Artificial Sequence
  Designed polypeptide
  misc_feature (38)..(38): X = Hyp (L-hydroxyproline)
RCNASTCTVNRLADQITQFSNKDKAQVSPPTEVGPNSX

SEQ ID NO: 10 - protein, 38 aa, Artificial Sequence
  Designed polypeptide
  misc_feature (38)..(38): X = Hyp (L-hydroxyproline)
KCNFATCTVQRLAHQIYQFTDKDKDNVAPPTEVGSNGX

SEQ ID NO: 11 - protein, 38 aa, Artificial Sequence
  Designed polypeptide
  misc_feature (38)..(38): X = Hyp (L-hydroxyproline)
KCNTATCTVQRLAHQINQFTDKDKDNVAPPTNVGSNGX

SEQ ID NO: 12 - protein, 38 aa, Artificial Sequence
  Designed polypeptide
  misc_feature (38)..(38): X = Hyp (L-hydroxyproline)
KCNTATCTVQRLAEQIYQFTDKDKDNKAPPTNVGSNGX

SEQ ID NO: 13 - protein, 38 aa, Artificial Sequence
  Designed polypeptide
  misc_feature (38)..(38): X = Hyp (L-hydroxyproline)
KCNTATCTVQRLAHAIYQFTDKDKDNVAPPTNVGSNGX

SEQ ID NO: 14 - protein, 38 aa, Artificial Sequence
  Designed polypeptide
  misc_feature (38)..(38): X = Hyp (L-hydroxyproline)
KCNTATCTVQRLAHQIAQFTDKDKDNVAPPTNVGSNGX

SEQ ID NO: 15 - protein, 38 aa, Artificial Sequence
  Designed polypeptide
  misc_feature (38)..(38): X = Hyp (L-hydroxyproline)
KCNTSTCTVARLADQITQFSDKDKANVSPPTEVGPNSX

SEQ ID NO: 16 - protein, 38 aa, Artificial Sequence
  Designed polypeptide
GCRFGTCTVQRLANFLYQFTDKDKDNVAPRTNVGPQGY

SEQ ID NO: 17 - protein, 38 aa, Artificial Sequence
  Designed polypeptide
  misc_feature (38)..(38): X = Hyp (L-hydroxyproline)
KCNFATCTVQRLAHQIYQFTDKDKDNVAPRTEVGSNGX

SEQ ID NO: 18 - protein, 38 aa, Artificial Sequence
  Designed polypeptide
KCNFATCTVQRLAHQIYQFTDKDKDNVAPPTEVGSNGP

SEQ ID NO: 19 - protein, 37 aa, Artificial Sequence
  Designed polypeptide
KCNTATCATQRLANFLVHSSNNFGAILPRTKVGSNGY

SEQ ID NO: 20 - protein, 38 aa, Artificial Sequence
  Designed polypeptide
  misc_feature (38)..(38): X = Hyp (L-hydroxyproline)
KCNTATCTVQRLAHQIYQFTDKDKDNVAPRTKVGSNGX

SEQ ID NO: 21 - protein, 38 aa, Artificial Sequence
  Designed polypeptide
  misc_feature (38)..(38): X = Hyp (L-hydroxyproline)
KCNTATCTVQRLANQIYQFTDKDKDNVAPPTNVGSNGX

SEQ ID NO: 22 - protein, 38 aa, Artificial Sequence
  Designed polypeptide
  misc_feature (38)..(38): X = Hyp (L-hydroxyproline)
KCNTATCTVQRLAHQITQFTDKDKDNVAPPTNVGSNGX

SEQ ID NO: 23 - protein, 38 aa, Artificial Sequence
  Designed polypeptide
  misc_feature (38)..(38): X = Hyp (L-hydroxyproline)
KCNTATCTVQRLAHQIYQFADKDKDNVAPPTNVGSNGX

SEQ ID NO: 24 - protein, 38 aa, Artificial Sequence
  Designed polypeptide
  misc_feature (38)..(38): X = Hyp (L-hydroxyproline)
KCNTATCTVQRLAHQIYQFTAKDKDNVAPPTNVGSNGX

SEQ ID NO: 25 - protein, 38 aa, Artificial Sequence
  Designed polypeptide
  misc_feature (38)..(38): X = Hyp (L-hydroxyproline)
KCNTATCTVQRLAHQIYQFTDKDADNVAPPTNVGSNGX

SEQ ID NO: 26 - protein, 38 aa, Artificial Sequence
  Designed polypeptide
  misc_feature (38)..(38): X = Hyp (L-hydroxyproline)
KCNTATCTVQRLAHQIYQFTDKDKANVAPPTNVGSNGX

SEQ ID NO: 27 - protein, 38 aa, Artificial Sequence
  Designed polypeptide
  misc_feature (38)..(38): X = Hyp (L-hydroxyproline)
KCNTATCTVQRLAHQIYQFTDKDKDNAAPPTNVGSNGX

SEQ ID NO: 28 - protein, 38 aa, Artificial Sequence
  Designed polypeptide
  misc_feature (38)..(38): X = Hyp (L-hydroxyproline)
KCNTATCTVQRLAHQIYQFTDKDKDNVAPATNVGSNGX

SEQ ID NO: 29 - protein, 37 aa, Artificial Sequence
  Designed polypeptide
  misc_feature (37)..(37): X = Hyp (L-hydroxyproline)
KCNTATCTVQRLAHQIYQFTKDKDNVAPPTNVGSNGX

SEQ ID NO: 30 - protein, 37 aa, Artificial Sequence
  Designed polypeptide
  misc_feature (37)..(37): X = Hyp (L-hydroxyproline)
KCNTATCTVQRLAHQIYQFTDKDKDNVPPTNVGSNGX

SEQ ID NO: 31 - protein, 37 aa, Artificial Sequence
  Designed polypeptide
  misc_feature (37)..(37): X = Hyp (L-hydroxyproline)
KCNTATCTVQRLAHQIYQFTDKDKDNVAPTNVGSNGX

SEQ ID NO: 32 - protein, 38 aa, Artificial Sequence
  Designed polypeptide
  misc_feature (38)..(38): X = Hyp (L-hydroxyproline)
RCQTSTCTVARLAEQIAQYTDKDKDQVAPPTNVGSNSX

SEQ ID NO: 33 - protein, 38 aa, Artificial Sequence
  Designed polypeptide
  misc_feature (11)..(11): X = Cit (L-citrulline)
  misc_feature (38)..(38): X = Hyp (L-hydroxyproline)
RCQASTCTVAXLAEQIAQYTDKDKDQVAPPTEVGPNSX

SEQ ID NO: 34 - protein, 38 aa, Artificial Sequence
  Designed polypeptide
KCNTATCTVQRLAHQIYQFTDKDKDNVAPRTKVGSNGY

SEQ ID NO: 35 - protein, 38 aa, Artificial Sequence
  Designed polypeptide
  misc_feature (38)..(38): X = Hyp (L-hydroxyproline)
KCNTATCTVQRLAHQIQQFTDKDKDNVAPPTNVGSNGX

SEQ ID NO: 36 - protein, 38 aa, Artificial Sequence
  Designed polypeptide
  misc_feature (38)..(38): X = Hyp (L-hydroxyproline)
KCKTATCTVQRLAEQIYQFTDKDKDNVAPPTNVGSNGX

SEQ ID NO: 37 - protein, 38 aa, Artificial Sequence
  Designed polypeptide
  misc_feature (38)..(38): X = Hyp (L-hydroxyproline)
KCNTATCTVARLAHQIYQFTDKDKDNVAPPTNVGSNGX

SEQ ID NO: 38 - protein, 38 aa, Artificial Sequence
  Designed polypeptide
  misc_feature (38)..(38): X = Hyp (L-hydroxyproline)
KCNTATCTVNRLAHQIYQFTDKDKDNVAPPTNVGSNGX

SEQ ID NO: 39 - protein, 38 aa, Artificial Sequence
  Designed polypeptide
  misc_feature (38)..(38): X = Hyp (L-hydroxyproline)
RCNTATCTVQRLAHQIYQFTDKDKDNVAPPTNVGSNGX

SEQ ID NO: 40 - protein, 38 aa, Artificial Sequence
  Designed polypeptide
  misc_feature (38)..(38): X = Hyp (L-hydroxyproline)
KCNTATCTVQRLAEQIYQFTDKDKKNVAPPTNVGSNGX

SEQ ID NO: 41 - protein, 38 aa, Artificial Sequence
  Designed polypeptide
  misc_feature (38)..(38): X = Hyp (L-hydroxyproline)
KCNTATCTVQRLAEQIYQFTDKDKDKVAPPTNVGSNGX

SEQ ID NO: 42 - protein, 38 aa, Artificial Sequence
  Designed polypeptide
  misc_feature (38)..(38): X = Hyp (L-hydroxyproline)
KCNTATCTVQRLAHQIYAFTDKDKDNVAPPTNVGSNGX

SEQ ID NO: 43 - protein, 38 aa, Artificial Sequence
  Designed polypeptide
  misc_feature (38)..(38): X = Hyp (L-hydroxyproline)
KCNTATCTVQRLAHQIYQFTDKAKDNVAPPTNVGSNGX

SEQ ID NO: 44 - protein, 38 aa, Artificial Sequence
  Designed polypeptide
  misc_feature (38)..(38): X = Hyp (L-hydroxyproline)
KCNTATCTVQRLAEQIYQFTDKDKDNVAPPYNEGSNGX

SEQ ID NO: 45 - protein, 38 aa, Artificial Sequence
  Designed polypeptide
  misc_feature (38)..(38): X = Hyp (L-hydroxyproline)
GCRFGTCTVQRLAHQIYQFTDKDKDNVAPRTKVGPQGX

SEQ ID NO: 46 - protein, 38 aa, Artificial Sequence
  Designed polypeptide
  misc_feature (38)..(38): X = Hyp (L-hydroxyproline)
GCRFGTCTVQRLAHQIYQFTDKDKDNVAPRTNIGPQGX

SEQ ID NO: 47 - protein, 38 aa, Artificial Sequence
  Designed polypeptide
  misc_feature (38)..(38): X = Hyp (L-hydroxyproline)
KCNTATCTVQRLAYQIYQFTDKDKDNVAPPTNVGSNGX

SEQ ID NO: 48 - protein, 38 aa, Artificial Sequence
  Designed polypeptide
  misc_feature (38)..(38): X = Hyp (L-hydroxyproline)
KCNTATCTVQRLAHQIYQYTDKDKDNVAPPTNVGSNGX

SEQ ID NO: 49 - protein, 38 aa, Artificial Sequence
  Designed polypeptide
  misc_feature (38)..(38): X = Hyp (L-hydroxyproline)
GCRTGTCTVQRLAHQIYQFTDKDKDNVAPRTNVGPQGX

SEQ ID NO: 50 - protein, 38 aa, Artificial Sequence
  Designed polypeptide
  misc_feature (38)..(38): X = Hyp (L-hydroxyproline)
KCNTSTCTVQRLAHQIYQFTDKDKDNVAPPTNVGSNGX

SEQ ID NO: 51 - protein, 38 aa, Artificial Sequence
  Designed polypeptide
  misc_feature (38)..(38): X = Hyp (L-hydroxyproline)
KCNTATCTVQRLAEQIYQFTDKDKDNVAPPTNVGSNGX

SEQ ID NO: 52 - protein, 38 aa, Artificial Sequence
  Designed polypeptide
  misc_feature (38)..(38): X = Hyp (L-hydroxyproline)
KCNTATCTVQRLAHQIYQFTDKDKDAVAPPTNVGSNGX

SEQ ID NO: 53 - protein, 38 aa, Artificial Sequence
  Designed polypeptide
  misc_feature (38)..(38): X = Hyp (L-hydroxyproline)
KCNTATCTVQRLAHQIYQFTDKDKDNVAAPTNVGSNGX

SEQ ID NO: 54 - protein, 38 aa, Artificial Sequence
  Designed polypeptide
GCRFGTCTVQRLAHFLYQFTDKDKDNVAPRTNVGPQGY

SEQ ID NO: 55 - protein, 38 aa, Artificial Sequence
  Designed polypeptide
  misc_feature (38)..(38): X = Hyp (L-hydroxyproline)
KCNTATCTVERLAHQIYQFTDKDKDNVAPPTNVGSNGX

SEQ ID NO: 56 - protein, 38 aa, Artificial Sequence
  Designed polypeptide
GCRFGTCTVQRLAHFLYQFTDKDKDNVAPRTNVGSNTY

SEQ ID NO: 57 - protein, 38 aa, Artificial Sequence
  Designed polypeptide
  misc_feature (38)..(38): X = Hyp (L-hydroxyproline)
KCNTATCTVQRLAHQIYQFSDKDKDNVAPPTNVGSNGX

SEQ ID NO: 58 - protein, 37 aa, Artificial Sequence
  Designed polypeptide
KCNTATCATQRLANFLVHSSNNFGAILSSTKVGSNTY

SEQ ID NO: 59 - protein, 37 aa, Artificial Sequence
  Designed polypeptide
KCNTATCATQRLANFLVHSSNNFGAILPSTKVGSNGY

SEQ ID NO: 60 - protein, 38 aa, Artificial Sequence
  Designed polypeptide
  misc_feature (38)..(38): X = Hyp (L-hydroxyproline)
KCNTATCTVQRLAHQIYQFTDKDKDNVAPPTKVGSNGX

SEQ ID NO: 61 - protein, 38 aa, Artificial Sequence; identical to SEQ ID NO: 14
  Designed polypeptide
  misc_feature (38)..(38): X = Hyp (L-hydroxyproline)

SEQ ID NO: 62 - protein, 38 aa, Artificial Sequence
  Designed polypeptide
  misc_feature (38)..(38): X = Hyp (L-hydroxyproline)
KCNTSTCTVQRLAHQIAQFTDKDKDNVAPPTNVGSNGX

SEQ ID NO: 63 - protein, 38 aa, Artificial Sequence
  Designed polypeptide
  misc_feature (38)..(38): X = Hyp (L-hydroxyproline)
KCNTATCTVQRLAEQIYQFTDKDKDNVAPPTAVGSNGX

SEQ ID NO: 64 - protein, 38 aa, Artificial Sequence
  Designed polypeptide
  misc_feature (38)..(38): X = Hyp (L-hydroxyproline)
KCNTATCTVQRLAHQIYQFTDADKDNVAPPTNVGSNGX

SEQ ID NO: 65 - protein, 37 aa, Artificial Sequence
  Designed polypeptide
  misc_feature (37)..(37): X = Hyp (L-hydroxyproline)
KCNTATCTVQRLAHQIYQFDKDKDNVAPPTNVGSNGX

SEQ ID NO: 66 - protein, 38 aa, Artificial Sequence
  Designed polypeptide
  misc_feature (38)..(38): X = Hyp (L-hydroxyproline)
KCNTATCTVQRLAEQIYQFTDKDKDNVSPPTNVGSNGX

SEQ ID NO: 67 - protein, 38 aa, Artificial Sequence; identical to SEQ ID NO: 17
  Designed polypeptide
  misc_feature (38)..(38): X = Hyp (L-hydroxyproline)

SEQ ID NO: 68 - protein, 38 aa, Artificial Sequence; identical to SEQ ID NO: 10
  Designed polypeptide
  misc_feature (38)..(38): X = Hyp (L-hydroxyproline)

SEQ ID NO: 69 - protein, 38 aa, Artificial Sequence
  Designed polypeptide
  misc_feature (38)..(38): X = Hyp (L-hydroxyproline)
KCNTATCTVQRLAHQIAQFTDKDKDNVAPPTNVGSNSX

SEQ ID NO: 70 - protein, 38 aa, Artificial Sequence
  Designed polypeptide
  misc_feature (38)..(38): X = Hyp (L-hydroxyproline)
GCRFGTCTVQRLAHQIYQFTDKDKDNVAPRTNVGPQGX

SEQ ID NO: 71 - protein, 38 aa, Artificial Sequence
  Designed polypeptide
  misc_feature (38)..(38): X = Hyp (L-hydroxyproline)
KCNTATCTVQRLAHQIAQYTDKDKDNVAPPTNVGSNGX

SEQ ID NO: 72 - protein, 38 aa, Artificial Sequence
  Designed polypeptide
  misc_feature (38)..(38): X = Hyp (L-hydroxyproline)
KCQTATCTVQRLAEQIYQFTDKDKDNVAPPTNVGSNGX

SEQ ID NO: 73 - protein, 38 aa, Artificial Sequence
  Designed polypeptide
  misc_feature (38)..(38): X = Hyp (L-hydroxyproline)
KCNTATCTVQRLAEQIYQFTDKDKDNVAPPTQVGSNGX

SEQ ID NO: 74 - protein, 38 aa, Artificial Sequence
  Designed polypeptide
  misc_feature (38)..(38): X = Hyp (L-hydroxyproline)
KCNTATCTVQRLAKQIYQFTDKDKDNVAPPTNVGSNGX

SEQ ID NO: 75 - protein, 38 aa, Artificial Sequence
  Designed polypeptide
  misc_feature (38)..(38): X = Hyp (L-hydroxyproline)
KCNTATCTVQRLAHQIYQFTDKDKDNVAPPTNVGSNGX

SEQ ID NO: 76 - protein, 35 aa, Artificial Sequence
  Designed polypeptide
  misc_feature (14)..(14): X = Aad (L-homoglutamic acid)
  misc_feature (22)..(22): X = Sar (Sarcosine)
  misc_feature (24)..(24): X = (NMe)I (N-methyl-L-isoleucine)
  misc_feature (35)..(35): X = Hyp (L-hydroxyproline)
RCGTATCATERLAXFLQRSSFXAXLSSTEVGSNTX

SEQ ID NO: 77 - protein, 38 aa, Artificial Sequence; identical to SEQ ID NO: 75
  Designed polypeptide
  misc_feature (38)..(38): X = Hyp (L-hydroxyproline)

SEQ ID NO: 78 - protein, 38 aa, Artificial Sequence
  Designed polypeptide
  misc_feature (38)..(38): X = Hyp (L-hydroxyproline)
KCNTATCTVQRLAEQIAQFTDKDKDNVAPPTNVGSNGX

SEQ ID NO: 79 - protein, 38 aa, Artificial Sequence
  Designed polypeptide
  misc_feature (38)..(38): X = Hyp (L-hydroxyproline)
KCNTATCTVQRLAHQIAQFSDKDKDNVAPPTNVGSNGX

SEQ ID NO: 80 - protein, 35 aa, Artificial Sequence
  Designed polypeptide
  misc_feature (22)..(22): X = Sar (Sarcosine)
  misc_feature (24)..(24): X = (NMe)I (N-methyl-L-isoleucine)
  misc_feature (35)..(35): X = Hyp (L-hydroxyproline)
RCQTATCATERLAHFLQRSSFXAXLSSTEVGSNTX

SEQ ID NO: 81 - protein, 38 aa, Artificial Sequence
  Designed polypeptide
  misc_feature (38)..(38): X = Hyp (L-hydroxyproline)
GCRFGTCTVQRLAHQIYQFTDKDKDNVAPRTNIGPNGX

SEQ ID NO: 82 - protein, 38 aa, Artificial Sequence
  Designed polypeptide
  misc_feature (38)..(38): X = Hyp (L-hydroxyproline)
KCNTATCTVQRLAHQIYQFTNKDKDNVAPPTNVGSNGX

SEQ ID NO: 83 - protein, 38 aa, Artificial Sequence; identical to SEQ ID NO: 23
  Designed polypeptide
  misc_feature (38)..(38): X = Hyp (L-hydroxyproline)

SEQ ID NO: 84 - protein, 38 aa, Artificial Sequence
  Designed polypeptide
GCRTGTCTVQRLAHQIYQFTDKDKDNVAPRTNVGPNGY

SEQ ID NO: 85 - protein, 38 aa, Artificial Sequence
  Designed polypeptide
  misc_feature (38)..(38): X = Hyp (L-hydroxyproline)
KCNTATCTVQRLAHQIVQFTDKDKDNVAPPTNVGSNGX

SEQ ID NO: 86 - protein, 38 aa, Artificial Sequence
  Designed polypeptide
  misc_feature (38)..(38): X = Hyp (L-hydroxyproline)
KCNTATCTVARLAHQINQFTDKDKDNVAPPTNVGSNGX

SEQ ID NO: 87 - protein, 38 aa, Artificial Sequence
  Designed polypeptide
  misc_feature (38)..(38): X = Hyp (L-hydroxyproline)
KCNTATCTVQRLAHQIAQFTDKNKDNVAPPTNVGSNGX

SEQ ID NO: 88 - protein, 38 aa, Artificial Sequence
  Designed polypeptide
  misc_feature (38)..(38): X = Hyp (L-hydroxyproline)
KCNTSTCTVQRLAHQIAQFTDKDKDPVAPPTNVGSNGX

SEQ ID NO: 89 - protein, 38 aa, Artificial Sequence
  Designed polypeptide
  misc_feature (38)..(38): X = Hyp (L-hydroxyproline)
KCNTATCTVQRLAEQIYQFKDKDKDNVAPPTNVGSNGX

SEQ ID NO: 90 - protein, 38 aa, Artificial Sequence
  Designed polypeptide
  misc_feature (38)..(38): X = Hyp (L-hydroxyproline)
GCRFGTCTVQRLAHQIYQFTDKDKDNVAPRTNVGPNGX

SEQ ID NO: 91 - protein, 38 aa, Artificial Sequence
  Designed polypeptide
  misc_feature (38)..(38): X = Hyp (L-hydroxyproline)
KCNTATCTVQRLAHQIYQFTDKNKDNVAPPTNVGSNGX

SEQ ID NO: 92 - protein, 38 aa, Artificial Sequence
  Designed polypeptide
  misc_feature (38)..(38): X = Hyp (L-hydroxyproline)
KCNTATCTVQRLAHQIAQFTDKDKDPVAPPTNVGSNGX

SEQ ID NO: 93 - protein, 37 aa, Artificial Sequence
  Designed polypeptide
KCNTATCATQRLANFLVHSSNNFGAIAPSTKVGSNGY

SEQ ID NO: 94 - protein, 38 aa, Artificial Sequence
  Designed polypeptide
  misc_feature (38)..(38): X = Hyp (L-hydroxyproline)
KCNTATCTVQRLAHQIAQFYDKDKDNVAPPTNVGSNGX

SEQ ID NO: 95 - protein, 38 aa, Artificial Sequence
  Designed polypeptide
  misc_feature (38)..(38): X = Hyp (L-hydroxyproline)
KCNTATCTVQRLAHQIAQFTNKDKDNVAPPTNVGSNGX

SEQ ID NO: 96 - protein, 38 aa, Artificial Sequence
  Designed polypeptide
  misc_feature (38)..(38): X = Hyp (L-hydroxyproline)
KCNTATCTVQRLAEQIYQFTDKDKDNVAPPTNVGSNTX

SEQ ID NO: 97 - protein, 38 aa, Artificial Sequence
  Designed polypeptide
  misc_feature (38)..(38): X = Hyp (L-hydroxyproline)
KCATATCTVQRLAEQIYQFTDKDKDNVAPPTNVGSNGX

SEQ ID NO: 98 - protein, 38 aa, Artificial Sequence
  Designed polypeptide
GCRFGTCTVQRLAHQIYQFTDKDKDNVAPRTNVSPNGY

SEQ ID NO: 99 - protein, 38 aa, Artificial Sequence; identical to SEQ ID NO: 20
  Designed polypeptide
  misc_feature (38)..(38): X = Hyp (L-hydroxyproline)

SEQ ID NO: 100 - protein, 38 aa, Artificial Sequence
  Designed polypeptide
  misc_feature (38)..(38): X = Hyp (L-hydroxyproline)
KCNTATCTVQRLAEQIYQFTDKDKDQVAPPTNVGSNGX

SEQ ID NO: 101 - protein, 38 aa, Artificial Sequence
  Designed polypeptide
  misc_feature (38)..(38): X = Hyp (L-hydroxyproline)
KCNAATCTVQRLAEQIYQFTDKDKDNVAPPTNVGSNGX

SEQ ID NO: 102 - protein, 38 aa, Artificial Sequence
  Designed polypeptide
KCNTATCTVQRLAHQIYQFTDKDKDNVAPRTEVGSNGY

SEQ ID NO: 103 - protein, 38 aa, Artificial Sequence
  Designed polypeptide
  misc_feature (38)..(38): X = Hyp (L-hydroxyproline)
KCNTATCTVVRLAHQIYQFTDKDKDNVAPPTNVGSNGX

SEQ ID NO: 104 - protein, 38 aa, Artificial Sequence
  Designed polypeptide
  misc_feature (38)..(38): X = Hyp (L-hydroxyproline)
KCNTATCTVQRLAHQIYQFYDKDKDNVAPPTNVGSNGX

SEQ ID NO: 105 - protein, 38 aa, Artificial Sequence
  Designed polypeptide
  misc_feature (38)..(38): X = Hyp (L-hydroxyproline)
KCNTATCTVQRLAHQIAQFADKDKDNVAPPTNVGSNGX

SEQ ID NO: 106 - protein, 38 aa, Artificial Sequence
  Designed polypeptide
  misc_feature (38)..(38): X = Hyp (L-hydroxyproline)
KCNTATCTVQRLAEQIYQFTAKDKDNVAPPTNVGSNGX

SEQ ID NO: 107 - protein, 38 aa, Artificial Sequence
  Designed polypeptide
  misc_feature (38)..(38): X = Hyp (L-hydroxyproline)
KCNTATCTVARLAHQIAQFTDKDKDNVAPPTNVGSNGX

SEQ ID NO: 108 - protein, 38 aa, Artificial Sequence
  Designed polypeptide
  misc_feature (38)..(38): X = Hyp (L-hydroxyproline)
KCNTATCTVQRLAEQIYQFTDKDKANVAPPTNVGSNGX

SEQ ID NO: 109 - protein, 38 aa, Artificial Sequence
  Designed polypeptide
GCRTGTCTVQRLAHQIYQFTDKDKDNVAPRTNVGPQGY

SEQ ID NO: 110 - protein, 38 aa, Artificial Sequence
  Designed polypeptide
  misc_feature (38)..(38): X = Hyp (L-hydroxyproline)
KCNTATCTVQRLAHQIEQFTDKDKDNVAPPTNVGSNGX

SEQ ID NO: 111 - protein, 38 aa, Artificial Sequence
  Designed polypeptide
  misc_feature (38)..(38): X = Hyp (L-hydroxyproline)
GCRFGTCTVQRLAHQIYQFTDKDKDNVAPRTKIGPQGX

SEQ ID NO: 112 - protein, 38 aa, Artificial Sequence
  Designed polypeptide
  misc_feature (38)..(38): X = Hyp (L-hydroxyproline)
KCNTATCTVDRLAHQIAQFTDKDKDNVAPPTNVGSNGX

SEQ ID NO: 113 - protein, 38 aa, Artificial Sequence
  Designed polypeptide
  misc_feature (38)..(38): X = Hyp (L-hydroxyproline)
GCRFGTCTVQRLAHQIYQFTDKDKDNVAPRTKISPNGX

SEQ ID NO: 114 - protein, 38 aa, Artificial Sequence
  Designed polypeptide
  misc_feature (38)..(38): X = Hyp (L-hydroxyproline)
KCNTATCTVQRLAHQIYQATDKDKDNVAPPTNVGSNGX

SEQ ID NO: 115 - protein, 38 aa, Artificial Sequence
  Designed polypeptide
  misc_feature (38)..(38): X = Hyp (L-hydroxyproline)
GCRTGTCTVQRLAHQIYQFTDKDKDNVAPRTKIGPNGX

SEQ ID NO: 116 - protein, 38 aa, Artificial Sequence
  Designed polypeptide
GCRFGTCTVQRLAHQIYQFTDKDKDNVAPRTNVSPQGY

SEQ ID NO: 117 - protein, 38 aa, Artificial Sequence
  Designed polypeptide
GCRFGTCTVQRLAHFLYQFTDKDKDNVAPRTKVGSNGY

SEQ ID NO: 118 - protein, 38 aa, Artificial Sequence
  Designed polypeptide
  misc_feature (38)..(38): X = Hyp (L-hydroxyproline)
GCRTGTCTVQRLAHQIYQFTDKDKDNVAPRTNIGPQGX

SEQ ID NO: 119 - protein, 38 aa, Artificial Sequence
  Designed polypeptide
  misc_feature (5)..(5): X = AIB (L-2-aminoisobutyric acid)
  misc_feature (38)..(38): X = Hyp (L-hydroxyproline)
KCNTXTCTVQRLAHQIYQFTDKDKDNVAPPTNVGSNGX

SEQ ID NO: 120 - protein, 38 aa, Artificial Sequence
  Designed polypeptide
  misc_feature (38)..(38): X = Hyp (L-hydroxyproline)
KCNTATCTVQRLAHQIAQFTDKDKDPVAPPTNVGSNSX

SEQ ID NO: 121 - protein, 38 aa, Artificial Sequence
  Designed polypeptide
  misc_feature (38)..(38): X = Hyp (L-hydroxyproline)
GCRTGTCTVQRLAHQIYQFTDKDKDNVAPRSNVGPQGX

SEQ ID NO: 122 - protein, 38 aa, Artificial Sequence
  Designed polypeptide
  misc_feature (38)..(38): X = Hyp (L-hydroxyproline)
KCNTATCTVQRLAEQIYQFTDKAKDNVAPPTNVGSNGX

SEQ ID NO: 123 - protein, 37 aa, Artificial Sequence
  Designed polypeptide
GCRFGTCTVQRLAHFLYQFTDKDGAIAPRTKIGSQGY

SEQ ID NO: 124 - protein, 38 aa, Artificial Sequence
  Designed polypeptide
  misc_feature (38)..(38): X = Hyp (L-hydroxyproline)
GCRFGTCTVQRLAHQIYQFTDKDKDNVAPRTKIGPNGX

SEQ ID NO: 125 - protein, 38 aa, Artificial Sequence
  Designed polypeptide
  misc_feature (38)..(38): X = Hyp (L-hydroxyproline)
GCRFGTCTVQRLAHQIYQFTDKDKDNVAPRTNVSPQGX

SEQ ID NO: 126 - protein, 38 aa, Artificial Sequence; identical to SEQ ID NO: 51
  Designed polypeptide
  misc_feature (38)..(38): X = Hyp (L-hydroxyproline)

SEQ ID NO: 127 - protein, 38 aa, Artificial Sequence
  Designed polypeptide
  misc_feature (38)..(38): X = Hyp (L-hydroxyproline)
GCRFGTCTVQRLAHQIYQFTDKDKDNVAPRSKIGPQGX

SEQ ID NO: 128 - protein, 37 aa, Artificial Sequence
  Designed polypeptide
KCNTATCATQRLANFLVHSSNNFGAIAPSTKIGPNGY

SEQ ID NO: 129 - protein, 38 aa, Artificial Sequence
  Designed polypeptide
GCRTGTCTVQRLAHQIYQFTDKDKDNVAPRSKVGPQGY

SEQ ID NO: 130 - protein, 38 aa, Artificial Sequence
  Designed polypeptide
  misc_feature (38)..(38): X = Hyp (L-hydroxyproline)
KCNTATCTVDRLAHQIAQFTDKDKDPVAPPTNVGSNGX

SEQ ID NO: 131 - protein, 38 aa, Artificial Sequence
  Designed polypeptide
GCRFGTCTVQRLAHQIYQFTDKDKDNVAPRSNVSPQGY

SEQ ID NO: 132 - protein, 38 aa, Artificial Sequence
  Designed polypeptide
  misc_feature (38)..(38): X = Hyp (L-hydroxyproline)
GCRFGTCTVQRLAHQIYQFTDKDKDNVAPRTKVSPQGX

SEQ ID NO: 133 - protein, 38 aa, Artificial Sequence
  Designed polypeptide
  misc_feature (38)..(38): X = Hyp (L-hydroxyproline)
KCNTATCTVARLAEQIYQFTDKDKDPVAPPTNVGSNGX

SEQ ID NO: 134 - protein, 38 aa, Artificial Sequence
  Designed polypeptide
  misc_feature (38)..(38): X = Hyp (L-hydroxyproline)
GCRFGTCTVQRLAHQIYQFTDKDKDNVAPRTKVSPNGX

SEQ ID NO: 135 - protein, 38 aa, Artificial Sequence
  Designed polypeptide
  misc_feature (38)..(38): X = Hyp (L-hydroxyproline)
GCRFGTCTVQRLAHQIYQFTDKDKDNVAPRSNVGPQGX

SEQ ID NO: 136 - protein, 38 aa, Artificial Sequence
  Designed polypeptide
  misc_feature (38)..(38): X = Hyp (L-hydroxyproline)
KCNTATCTVQRLAEQIKQFTDKDKDNVAPPTNVGSNGX

SEQ ID NO: 137 - protein, 38 aa, Artificial Sequence
  Designed polypeptide
  misc_feature (38)..(38): X = Hyp (L-hydroxyproline)
KCNTATCTVARLAHQINQFTDKDKDPVAPPTNVGSNGX

SEQ ID NO: 138 - protein, 38 aa, Artificial Sequence
  Designed polypeptide
GCRTGTCTVQRLAHQIYQFTDKDKDNVAPRSNVGPQGY

SEQ ID NO: 139 - protein, 38 aa, Artificial Sequence
  Designed polypeptide
  misc_feature (38)..(38): X = Hyp (L-hydroxyproline)
GCRTGTCTVQRLAHQIYQFTDKDKDNVAPRSKVGPNGX

SEQ ID NO: 140 - protein, 38 aa, Artificial Sequence
  Designed polypeptide
GCRFGTCTVQRLAHQIYQFTDKDKDNVAPRTNISPQGY

SEQ ID NO: 141 - protein, 38 aa, Artificial Sequence
  Designed polypeptide
  misc_feature (38)..(38): X = Hyp (L-hydroxyproline)
GCRFGTCTVQRLAHQIYQFTDKDKDNVAPRTNISPQGX

SEQ ID NO: 142 - protein, 38 aa, Artificial Sequence
  Designed polypeptide
GCRTGTCTVQRLAHQIYQFTDKDKDNVAPRTNIGPNGY

SEQ ID NO: 143 - protein, 38 aa, Artificial Sequence
  Designed polypeptide
  misc_feature (38)..(38): X = Hyp (L-hydroxyproline)
GCRTGTCTVQRLAHQIYQFTDKDKDNVAPRTKVGPQGX

SEQ ID NO: 144 - protein, 38 aa, Artificial Sequence
  Designed polypeptide
  misc_feature (38)..(38): X = Hyp (L-hydroxyproline)
KCNTATCTVQRLAEQIAQFTDKDKDPVAPPTNVGSNGX

SEQ ID NO: 145 - protein, 38 aa, Artificial Sequence
  Designed polypeptide
  misc_feature (38)..(38): X = Hyp (L-hydroxyproline)
GCRFGTCTVQRLAHQIYQFTDKDKDNVAPRSNVSPQGX

SEQ ID NO: 146 - protein, 38 aa, Artificial Sequence
  Designed polypeptide
  misc_feature (38)..(38): X = Hyp (L-hydroxyproline)
GCRFGTCTVQRLAHQIYQFTDKDKDNVAPRTKISPQGX

SEQ ID NO: 147 - protein, 38 aa, Artificial Sequence
  Designed polypeptide
  misc_feature (38)..(38): X = Hyp (L-hydroxyproline)
GCRIGTCTVQRLAHQIYQFTDKFKDNVAPRSKISPQTX

SEQ ID NO: 148 - protein, 37 aa, Artificial Sequence
  Designed polypeptide
KCNTATCATQRLANFLVHSSNNFGAILSSTKIGSNGY

SEQ ID NO: 149 - protein, 37 aa, Artificial Sequence
  Designed polypeptide
KCNTATCATQRLANFLVHSSNNFGAILPSTKVGPNGY

SEQ ID NO: 150 - protein, 38 aa, Artificial Sequence
  Designed polypeptide
  misc_feature (38)..(38): X = Hyp (L-hydroxyproline)
GCRWGTCTVQRLAHQIYQFTDKDKDNVAPRSKISPQTX

SEQ ID NO: 151 - protein, 38 aa, Artificial Sequence
  Designed polypeptide
  misc_feature (38)..(38): X = Hyp (L-hydroxyproline)
GCRTGTCTVQRLAHQIYQFTDKDKDNVAPRSNIGPNGX

SEQ ID NO: 152 - protein, 38 aa, Artificial Sequence
  Designed polypeptide
  misc_feature (38)..(38): X = Hyp (L-hydroxyproline)
GCRFGTCTVQRLAHQIYQFTDKDKDNVAPRSKVGPQGX

SEQ ID NO: 153 - protein, 38 aa, Artificial Sequence
  Designed polypeptide
  misc_feature (11)..(11): X = Cit (L-citrulline)
  misc_feature (38)..(38): X = Hyp (L-hydroxyproline)
KCNTATCTVQXLAEQIAQFTDKDKDNVAPPTNVGSNGX

SEQ ID NO: 154 - protein, 38 aa, Artificial Sequence
  Designed polypeptide
GCRFGTCTVQRLAHQIYQFTDKDKDNVAPRSKISPQGY

SEQ ID NO: 155 - protein, 38 aa, Artificial Sequence
  Designed polypeptide
GCRFGTCTVQRLAHQIYQFTDKDKDNVAPRTKVSPQGY

SEQ ID NO: 156 - protein, 38 aa, Artificial Sequence
  Designed polypeptide
GCRTGTCTVQRLAHQIYQFTDKDKDNVAPRTKVGPQGY

SEQ ID NO: 157 - protein, 38 aa, Artificial Sequence
  Designed polypeptide
  misc_feature (38)..(38): X = Hyp (L-hydroxyproline)
GCRTGTCTVQRLAHQIYQFTDKDKDNVAPRSKIGPNGX

SEQ ID NO: 158 - protein, 38 aa, Artificial Sequence
  Designed polypeptide
  misc_feature (38)..(38): X = Hyp (L-hydroxyproline)
GCRFGTCTVQRLAHQIYQFTDKDKDNVAPRSNISPQGX

SEQ ID NO: 159 - protein, 38 aa, Artificial Sequence
  Designed polypeptide
  misc_feature (38)..(38): X = Hyp (L-hydroxyproline)
KCNTATCTVIRLAHQIYQFTDKDKDNVAPPTNVGSNGX

SEQ ID NO: 160 - protein, 38 aa, Artificial Sequence
  Designed polypeptide
GCRTGTCTVQRLAHQIYQFTDKDKDNVAPRTNIGPQGY

SEQ ID NO: 161 - protein, 38 aa, Artificial Sequence
  Designed polypeptide
  misc_feature (38)..(38): X = Hyp (L-hydroxyproline)
GCRTGTCTVQRLAHQIYQFTDKDKDNVAPRTKIGPQGX

SEQ ID NO: 162 - protein, 37 aa, Artificial Sequence
  Designed polypeptide
KCNTATCATQRLANFLVHSSNNFGAILPSTKIGPNGY

SEQ ID NO: 163 - protein, 38 aa, Artificial Sequence
  Designed polypeptide
  misc_feature (38)..(38): X = Hyp (L-hydroxyproline)
GCRTGTCTVQRLAHQIYQFTDKDKDNVAPRTNVSPNGX

SEQ ID NO: 164 - protein, 38 aa, Artificial Sequence
  Designed polypeptide
GCRFGTCTVQRLAHQIYQFTDKDKDNVAPRTKISPQGY

SEQ ID NO: 165 - protein, 38 aa, Artificial Sequence
  Designed polypeptide
  misc_feature (38)..(38): X = Hyp (L-hydroxyproline)
GCRTGTCTVQRLAHQIYQFTDKDKDNVAPRSNIGPQGX

SEQ ID NO: 166 - protein, 38 aa, Artificial Sequence
  Designed polypeptide
  misc_feature (38)..(38): X = Hyp (L-hydroxyproline)
GCRTGTCTVQRLAHQIYQFTDKDKDNVAPRSNVSPNGX

SEQ ID NO: 167 - protein, 38 aa, Artificial Sequence
  Designed polypeptide
  misc_feature (38)..(38): X = Hyp (L-hydroxyproline)
GCRFGTCTVQRLAHQIYQFTDKDKDNVAPRSKVSPQGX

SEQ ID NO: 168 - protein, 38 aa, Artificial Sequence
  Designed polypeptide
  misc_feature (38)..(38): X = Hyp (L-hydroxyproline)
GCRFGTCTVQRLAHQIYQFTDKDKDNVAPRSKISPQTX

SEQ ID NO: 169 - protein, 38 aa, Artificial Sequence
  Designed polypeptide
  misc_feature (38)..(38): X = Hyp (L-hydroxyproline)
GCRFGTCTVQRLAHQIYQFTDKDKDNVAPRSKISPQGX

SEQ ID NO: 170 - protein, 38 aa, Artificial Sequence
  Designed polypeptide
  misc_feature (38)..(38): X = Hyp (L-hydroxyproline)
GCRTGTCTVQRLAHQIYQFTDKDKDNVAPRTNISPNGX

SEQ ID NO: 171 - protein, 38 aa, Artificial Sequence
  Designed polypeptide
  misc_feature (38)..(38): X = Hyp (L-hydroxyproline)
GCRWGTCTVQRLAHQIYQFTDKFKDNVAPRSKISPQTX

SEQ ID NO: 172 - protein, 38 aa, Artificial Sequence
  Designed polypeptide
GCRTGTCTVQRLAHQIYQFTDKDKDNVAPRSNVSPNGY

SEQ ID NO: 173 - protein, 38 aa, Artificial Sequence
  Designed polypeptide
  misc_feature (38)..(38): X = Hyp (L-hydroxyproline)
GCRMGTCTVQRLAHQIYQFTDKFKDNVAPRSKISPQTX

SEQ ID NO: 174 - protein, 38 aa, Artificial Sequence
  Designed polypeptide
GCRFGTCTVQRLAHQIYQFTDKDKDNVAPRSKVSPQGY

SEQ ID NO: 175 - protein, 38 aa, Artificial Sequence
  Designed polypeptide
  misc_feature (38)..(38): X = Hyp (L-hydroxyproline)
GCRFGTCTVQRLAHQIYQFTDKDKDNVAPRSKVSPNGX

SEQ ID NO: 176 - protein, 38 aa, Artificial Sequence
  Designed polypeptide
GCRTGTCTVQRLAHQIYQFTDKDKDNVAPRTNVSPQGY

SEQ ID NO: 177 - protein, 38 aa, Artificial Sequence
  Designed polypeptide
GCRTGTCTVQRLAHQIYQFTDKDKDNVAPRSNVGPNGY

SEQ ID NO: 178 - protein, 38 aa, Artificial Sequence
  Designed polypeptide
  misc_feature (38)..(38): X = Hyp (L-hydroxyproline)
GCRTGTCTVQRLAHQIYQFTDKDKDNVAPRTNVSPQGX

SEQ ID NO: 179 - protein, 38 aa, Artificial Sequence
  Designed polypeptide
  misc_feature (38)..(38): X = Hyp (L-hydroxyproline)
GCRTGTCTVQRLAHQIYQFTDKDKDNVAPRSKIGPQGX

SEQ ID NO: 180 - protein, 37 aa, Artificial Sequence
  Designed polypeptide
KCNTATCATQRLANFLVHSSNNFGAILPSTKIGSNTY

SEQ ID NO: 181 - protein, 37 aa, Artificial Sequence
  Designed polypeptide
  misc_feature (37)..(37): X = Hyp (L-hydroxyproline)
KCNTATCTVQRLAHQIYFTDKDKDNVAPPTNVGSNGX

SEQ ID NO: 182 - protein, 38 aa, Artificial Sequence
  Designed polypeptide
GCRFGTCTVQRLAHQIYQFTDKDKDNVAPRSNISPQGY

SEQ ID NO: 183 - protein, 38 aa, Artificial Sequence
  Designed polypeptide
GCRTGTCTVQRLAHQIYQFTDKDKDNVAPRSNVSPQGY

SEQ ID NO: 184 - protein, 38 aa, Artificial Sequence
  Designed polypeptide
GCRTGTCTVQRLAHQIYQFTDKFKDNVAPRSKISPQTW

SEQ ID NO: 185 - protein, 38 aa, Artificial Sequence
  Designed polypeptide
  misc_feature (38)..(38): X = Hyp (L-hydroxyproline)
GCRTGTCTVQRLAHQIYQFTDKFKDNVAPRSKISPQWX

SEQ ID NO: 186 - protein, 38 aa, Artificial Sequence
  Designed polypeptide
  misc_feature (38)..(38): X = Hyp (L-hydroxyproline)
GCRTGTCTVQRLAHQIYQFTDKFKDNVAPRSKISPQYX

SEQ ID NO: 187 - protein, 38 aa, Artificial Sequence
  Designed polypeptide
  misc_feature (38)..(38): X = Hyp (L-hydroxyproline)
GCRTGTCTVQRLAHQIYQFTDKDKDNVAPRSKVGPQGX

SEQ ID NO: 188 - protein, 38 aa, Artificial Sequence
  Designed polypeptide
GCRTGTCTVQRLAHQIYQFTDKDKDNVAPRTNISPNGY

SEQ ID NO: 189 - protein, 38 aa, Artificial Sequence
  Designed polypeptide
  misc_feature (38)..(38): X = Hyp (L-hydroxyproline)
GCRTGTCTVQRLAHQIYQFTDKDKDNVAPRTKISPQGX

SEQ ID NO: 190 - protein, 38 aa, Artificial Sequence
  Designed polypeptide
GCRTGTCTVQRLAHQIYQFTDKDKDNVAPRTKISPNGY

SEQ ID NO: 191 - protein, 38 aa, Artificial Sequence
  Designed polypeptide
GCRTGTCTVQRLAHQIYQFTDKDKDNVAPRSNIGPQGY

SEQ ID NO: 192 - protein, 38 aa, Artificial Sequence
  Designed polypeptide
  misc_feature (38)..(38): X = Hyp (L-hydroxyproline)
GCRMGTCTVQRLAHQIYQFTNKDKDNVAPRSKISPQTX

SEQ ID NO: 193 - protein, 38 aa, Artificial Sequence
  Designed polypeptide
  misc_feature (38)..(38): X = Hyp (L-hydroxyproline)
GCRTGTCTVQRLAHQIHQFTDKFKDNVAPRSKISPQTX

SEQ ID NO: 194 - protein, 38 aa, Artificial Sequence
  Designed polypeptide
  misc_feature (38)..(38): X = Hyp (L-hydroxyproline)
KCRMGTCTVQRLAHQIYQFTDKDKDNVAPRSKISPQTX

SEQ ID NO: 195 - protein, 37 aa, Artificial Sequence
  Designed polypeptide
  misc_feature (37)..(37): X = Hyp (L-hydroxyproline)
KCNTATCTVQRLAHQIYQTDKDKDNVAPPTNVGSNGX

SEQ ID NO: 196 - protein, 38 aa, Artificial Sequence
  Designed polypeptide
  misc_feature (38)..(38): X = Hyp (L-hydroxyproline)
GCRTGTCTVQRLAHQIAQFTDKFKDNVAPRSKISPQTX

SEQ ID NO: 197 - protein, 38 aa, Artificial Sequence
  Designed polypeptide
  misc_feature (38)..(38): X = Hyp (L-hydroxyproline)
GCRTGTCTVQRLAHQIYQFTDKDKDNVAPRTKISPNGX

SEQ ID NO: 198 - protein, 38 aa, Artificial Sequence
  Designed polypeptide
  misc_feature (38)..(38): X = Hyp (L-hydroxyproline)
GCRIGTCTVQRLAHQIYQFTNKDKDNVAPRSKISPQTX

SEQ ID NO: 199 - protein, 38 aa, Artificial Sequence
  Designed polypeptide
GCRTGTCTVQRLAHQIYQFTDKDKDNVAPRTNISPQGY

SEQ ID NO: 200 - protein, 38 aa, Artificial Sequence; identical to SEQ ID NO: 54
  Designed polypeptide

SEQ ID NO: 201 - protein, 38 aa, Artificial Sequence
  Designed polypeptide
  misc_feature (38)..(38): X = Hyp (L-hydroxyproline)
GCRTGTCTVQRLAHQIYQFTDKFKDNVAPRSKISPQHX

SEQ ID NO: 202 - protein, 38 aa, Artificial Sequence
  Designed polypeptide
  misc_feature (38)..(38): X = Hyp (L-hydroxyproline)
GCRWGTCTVQRLAHQIYQFTDKDKDNVAPSSKISPQTX

SEQ ID NO: 203 - protein, 38 aa, Artificial Sequence
  Designed polypeptide
  misc_feature (38)..(38): X = Hyp (L-hydroxyproline)
GCRTGTCTVQRLAHQIYQFTDKFKDNVAPRSKISPQPX

SEQ ID NO: 204 - protein, 38 aa, Artificial Sequence
  Designed polypeptide
  misc_feature (38)..(38): X = Hyp (L-hydroxyproline)
GCRTGTCTVQRLAHQIYQFTDKDKDNVAPRSKVSPNGX

SEQ ID NO: 205 - protein, 38 aa, Artificial Sequence
  Designed polypeptide
  misc_feature (38)..(38): X = Hyp (L-hydroxyproline)
KCRFGTCTVQRLAHQIYQFTDKDKDNVAPRSKISPQTX

SEQ ID NO: 206 - protein, 38 aa, Artificial Sequence
  Designed polypeptide
  misc_feature (38)..(38): X = Hyp (L-hydroxyproline)
GCRTGTCTVQRLAHQIYQFTDKFKDNVAPRSKISPQKX

SEQ ID NO: 207 - protein, 37 aa, Artificial Sequence
  Designed polypeptide
KCNTATCATQRLANFLVHSSNNFGAILPSTKIGSNGY

SEQ ID NO: 208 - protein, 38 aa, Artificial Sequence; identical to SEQ ID NO: 56
  Designed polypeptide

SEQ ID NO: 209 - protein, 38 aa, Artificial Sequence
  Designed polypeptide
GCRTGTCTVQRLAHQIYQFTDKDKDNVAPRTKVSPQGY

SEQ ID NO: 210 - protein, 38 aa, Artificial Sequence
  Designed polypeptide
  misc_feature (38)..(38): X = Hyp (L-hydroxyproline)
KCNTATCTVQRLAHQAYQFTDKDKDNVAPPTNVGSNGX

SEQ ID NO: 211 - protein, 38 aa, Artificial Sequence
  Designed polypeptide
  misc_feature (38)..(38): X = Hyp (L-hydroxyproline)
GCRTGTCTVQRLAHQIYQFTDKFKDNVAPRSKISPQFX

SEQ ID NO: 212 - protein, 38 aa, Artificial Sequence
  Designed polypeptide
  misc_feature (38)..(38): X = Hyp (L-hydroxyproline)
GCRFGTCTVQRLAHQIYQFTDKFKDNVAPRSKISPQTX

SEQ ID NO: 213 - protein, 38 aa, Artificial Sequence
  Designed polypeptide
  misc_feature (38)..(38): X = Hyp (L-hydroxyproline)
GCRTGTCTVQRLAHQIWQFTDKFKDNVAPRSKISPQTX

SEQ ID NO: 214 - protein, 38 aa, Artificial Sequence
  Designed polypeptide
  misc_feature (38)..(38): X = Hyp (L-hydroxyproline)
GCRTGTCTVQRLAHQIYQFTDKDKDNVAPRTNISPQGX

SEQ ID NO: 215 - protein, 38 aa, Artificial Sequence
  Designed polypeptide
GCRTGTCTVQRLAHQIYQFTDKFKDNVAPRSKISPQTM

SEQ ID NO: 216 - protein, 38 aa, Artificial Sequence
  Designed polypeptide
  misc_feature (38)..(38): X = Hyp (L-hydroxyproline)
GCRTGTCTVQRLAHQIYQFTDKDKDNVAPRTKVSPQGX

SEQ ID NO: 217 - protein, 38 aa, Artificial Sequence
  Designed polypeptide
  misc_feature (38)..(38): X = Hyp (L-hydroxyproline)
GCRFGTCTVQRLAHQLYQFTDKDKDNVAPRSKISPQTX

SEQ ID NO: 218 - protein, 38 aa, Artificial Sequence
  Designed polypeptide
  misc_feature (38)..(38): X = Hyp (L-hydroxyproline)
GCRTGTCTVQRLAHQIYQFTDKFKDNVAPRSKISPQAX

SEQ ID NO: 219 - protein, 38 aa, Artificial Sequence
  Designed polypeptide
  misc_feature (38)..(38): X = Hyp (L-hydroxyproline)
GCRTGTCTVQRLAHQIYQFTNKDKDNVAPRSKISPQHX

SEQ ID NO: 220 - protein, 38 aa, Artificial Sequence
  Designed polypeptide
  misc_feature (38)..(38): X = Hyp (L-hydroxyproline)
GCRTGTCTVQRLAHQIYQFTNKDKDNVAPRSKISPQWX

SEQ ID NO: 221 - protein, 38 aa, Artificial Sequence; identical to SEQ ID NO: 51
  Designed polypeptide
  misc_feature (38)..(38): X = Hyp (L-hydroxyproline)

SEQ ID NO: 222 - protein, 38 aa, Artificial Sequence
  Designed polypeptide
  misc_feature (38)..(38): X = Hyp (L-hydroxyproline)
GCRMGTCTVQRLAHQIYQFTDKDKDNVAPSSKISPQTX

SEQ ID NO: 223 - protein, 38 aa, Artificial Sequence; identical to SEQ ID NO: 117
  Designed polypeptide

SEQ ID NO: 224 - protein, 38 aa, Artificial Sequence
  Designed polypeptide
  misc_feature (38)..(38): X = Hyp (L-hydroxyproline)
GCRTGTCTVQRLAHQIYQFTDKDKDNVAPRSNVSPQGX

SEQ ID NO: 225 - protein, 38 aa, Artificial Sequence
  Designed polypeptide
  misc_feature (38)..(38): X = Hyp (L-hydroxyproline)
KCNTLTCTVQRLAHQIYQFTDKDKDNVAPPTNVGSNGX

SEQ ID NO: 226 - protein, 38 aa, Artificial Sequence
  Designed polypeptide
GCRTGTCTVQRLAHQIYQFTNKDKDNVAPRSKISPQTW

SEQ ID NO: 227 - protein, 38 aa, Artificial Sequence
  Designed polypeptide
  misc_feature (38)..(38): X = Hyp (L-hydroxyproline)
GCRTGTCTVQRLAHQIHQFTNKDKDNVAPRSKISPQTX

SEQ ID NO: 228 - protein, 38 aa, Artificial Sequence
  Designed polypeptide
  misc_feature (38)..(38): X = Hyp (L-hydroxyproline)
GCRTGTCTVQRLAHQIHQFTDKDKDNVAPRSKISPQTX

SEQ ID NO: 229 - protein, 38 aa, Artificial Sequence
  Designed polypeptide
  misc_feature (38)..(38): X = Hyp (L-hydroxyproline)
GCRFGTCTVQRLAHQIYQFTDKDKDNVAPRSNIGPQGX

SEQ ID NO: 230 - protein, 38 aa, Artificial Sequence
  Designed polypeptide
GCRTGTCTVQRLAHQIYQFTDKFKDNVAPRSKISPQTY

SEQ ID NO: 231 - protein, 38 aa, Artificial Sequence
  Designed polypeptide
  misc_feature (38)..(38): X = Hyp (L-hydroxyproline)
KCNTYTCTVQRLAHQIYQFTDKDKDNVAPPTNVGSNGX

SEQ ID NO: 232 - protein, 38 aa, Artificial Sequence
  Designed polypeptide
  misc_feature (38)..(38): X = Hyp (L-hydroxyproline)
GCRTGTCTVQRLAHQIYQFTNKDKDNVAPRSKISPQQX

SEQ ID NO: 233 - protein, 38 aa, Artificial Sequence; identical to SEQ ID NO: 51
  Designed polypeptide
  misc_feature (38)..(38): X = Hyp (L-hydroxyproline)

SEQ ID NO: 234 - protein, 38 aa, Artificial Sequence
  Designed polypeptide
KCNTATCATQRLANFLVQFTDKDKDNVAPRSKISPQGY

SEQ ID NO: 235 - protein, 38 aa, Artificial Sequence
  Designed polypeptide
GCRTGTCTVQRLAHQIYQFTDKFKDNVAPRSKISPQTP

SEQ ID NO: 236 - protein, 38 aa, Artificial Sequence
  Designed polypeptide
  misc_feature (38)..(38): X = Hyp (L-hydroxyproline)
GCRTGTCTVQRLAHQIYQFTDKFKDNVAPRSKISPQMX

SEQ ID NO: 237 - protein, 38 aa, Artificial Sequence
  Designed polypeptide
GCRTGTCTVQRLAHQIYQFTNKDKDNVAPRSKISPQTM

SEQ ID NO: 238 - protein, 38 aa, Artificial Sequence
  Designed polypeptide
  misc_feature (38)..(38): X = Hyp (L-hydroxyproline)
GCRTGTCTVQRLAHQIYQFTNKDKDNVAPRSKISPQFX

SEQ ID NO: 239 - protein, 38 aa, Artificial Sequence
  Designed polypeptide
GCRTGTCTVQRLAHQIYQFTDKFKDNVAPRSKISPQTF

SEQ ID NO: 240 - protein, 38 aa, Artificial Sequence
  Designed polypeptide
  misc_feature (38)..(38): X = Hyp (L-hydroxyproline)
GCRFGTCTVQRLAHQIYQFTDKDKDNVAPSSKISPQTX

SEQ ID NO: 241 - protein, 38 aa, Artificial Sequence
  Designed polypeptide
GCRTGTCTVQRLAHQIYQFTDKFKDNVAPRSKISPQTA

SEQ ID NO: 242 - protein, 38 aa, Artificial Sequence
  Designed polypeptide
GCRTGTCTVQRLAHQIYQFTNKDKDNVAPRSKISPQTR

SEQ ID NO: 243 - protein, 38 aa, Artificial Sequence
  Designed polypeptide
  misc_feature (11)..(11): X = Cit (L-citrulline)
  misc_feature (38)..(38): X = Hyp (L-hydroxyproline)
KCNTATCTVQXLAAQIYQFTDKDKDNVAPPTNVGSNGX

SEQ ID NO: 244 - protein, 38 aa, Artificial Sequence
  Designed polypeptide
  misc_feature (11)..(11): X = Cit (L-citrulline)
  misc_feature (38)..(38): X = Hyp (L-hydroxyproline)
KCNTSTCTVAXLADQITQFSNKDKAQVSPPTEVGPNSX

SEQ ID NO: 245 - protein, 38 aa, Artificial Sequence
  Designed polypeptide
  misc_feature (11)..(11): X = Cit (L-citrulline)
  misc_feature (38)..(38): X = Hyp (L-hydroxyproline)
RCNASTCTVNXLADQITQFSNKDKAQVSPPTEVGPNSX

SEQ ID NO: 246 - protein, 38 aa, Artificial Sequence
  Designed polypeptide
  misc_feature (11)..(11): X = Cit (L-citrulline)
  misc_feature (38)..(38): X = Hyp (L-hydroxyproline)
KCNTATCTVQXLAHQIAQFTDKDKDNVAPPTNVGSNGX

SEQ ID NO: 247 - protein, 38 aa, Artificial Sequence
  Designed polypeptide
  misc_feature (11)..(11): X = Cit (L-citrulline)
  misc_feature (38)..(38): X = Hyp (L-hydroxyproline)
KCNTSTCTVAXLADQITQFSDKDKANVSPPTEVGPNSX

SEQ ID NO: 248 - protein, 38 aa, Artificial Sequence
  Designed polypeptide
  misc_feature (11)..(11): X = Cit (L-citrulline)
  misc_feature (38)..(38): X = Hyp (L-hydroxyproline)
KCNTATCTVQXLAHQIYQFTDKDKDNVAPRTKVGSNGX

SEQ ID NO: 249 - protein, 38 aa, Artificial Sequence
  Designed polypeptide
  misc_feature (11)..(11): X = Cit (L-citrulline)
  misc_feature (38)..(38): X = Hyp (L-hydroxyproline)
KCNTATCTVQXLAHQIYQFADKDKDNVAPPTNVGSNGX

SEQ ID NO: 250 - protein, 38 aa, Artificial Sequence
  Designed polypeptide
  misc_feature (11)..(11): X = Cit (L-citrulline)
  misc_feature (38)..(38): X = Hyp (L-hydroxyproline)
KCNTATCTVQXLAHQIYQFTDKDADNVAPPTNVGSNGX

SEQ ID NO: 251 - protein, 38 aa, Artificial Sequence
  Designed polypeptide
  misc_feature (11)..(11): X = Cit (L-citrulline)
  misc_feature (38)..(38): X = Hyp (L-hydroxyproline)
KCNTATCTVQXLAHQIYQFTDKDKDNAAPPTNVGSNGX

SEQ ID NO: 252 - protein, 38 aa, Artificial Sequence
  Designed polypeptide
  misc_feature (11)..(11): X = Cit (L-citrulline)
  misc_feature (38)..(38): X = Hyp (L-hydroxyproline)
KCNTATCTVQXLAHQIYQFTDKDKDNVAPATNVGSNGX

SEQ ID NO: 253 - protein, 37 aa, Artificial Sequence
  Designed polypeptide
  misc_feature (11)..(11): X = Cit (L-citrulline)
  misc_feature (37)..(37): X = Hyp (L-hydroxyproline)
KCNTATCTVQXLAHQIYQFTKDKDNVAPPTNVGSNGX

SEQ ID NO: 254 - protein, 37 aa, Artificial Sequence
  Designed polypeptide
  misc_feature (11)..(11): X = Cit (L-citrulline)
  misc_feature (37)..(37): X = Hyp (L-hydroxyproline)
KCNTATCTVQXLAHQIYQFTDKDKDNVPPTNVGSNGX

SEQ ID NO: 255 - protein, 37 aa, Artificial Sequence
  Designed polypeptide
  misc_feature (11)..(11): X = Cit (L-citrulline)
  misc_feature (37)..(37): X = Hyp (L-hydroxyproline)
KCNTATCTVQXLAHQIYQFTDKDKDNVAPTNVGSNGX

SEQ ID NO: 256 - protein, 38 aa, Artificial Sequence
  Designed polypeptide
  misc_feature (11)..(11): X = Cit (L-citrulline)
  misc_feature (38)..(38): X = Hyp (L-hydroxyproline)
RCQTSTCTVAXLAEQIAQYTDKDKDQVAPPTNVGSNSX

SEQ ID NO: 257 - protein, 38 aa, Artificial Sequence
  Designed polypeptide
  misc_feature (11)..(11): X = Cit (L-citrulline)
KCNTATCTVQXLAHQIYQFTDKDKDNVAPRTKVGSNGY

SEQ ID NO: 258 - protein, 38 aa, Artificial Sequence
  Designed polypeptide
  misc_feature (11)..(11): X = Cit (L-citrulline)
  misc_feature (38)..(38): X = Hyp (L-hydroxyproline)
KCNTATCTVQXLAHQIYQFTDKAKDNVAPPTNVGSNGX

SEQ ID NO: 259 - protein, 38 aa, Artificial Sequence
  Designed polypeptide
  misc_feature (11)..(11): X = Cit (L-citrulline)
  misc_feature (38)..(38): X = Hyp (L-hydroxyproline)
GCRFGTCTVQXLAHQIYQFTDKDKDNVAPRTKVGPQGX

SEQ ID NO: 260 - protein, 38 aa, Artificial Sequence
  Designed polypeptide
  misc_feature (11)..(11): X = Cit (L-citrulline)
  misc_feature (38)..(38): X = Hyp (L-hydroxyproline)
GCRFGTCTVQXLAHQIYQFTDKDKDNVAPRTNIGPQGX

SEQ ID NO: 261 - protein, 38 aa, Artificial Sequence
  Designed polypeptide
  misc_feature (11)..(11): X = Cit (L-citrulline)
  misc_feature (38)..(38): X = Hyp (L-hydroxyproline)
GCRTGTCTVQXLAHQIYQFTDKDKDNVAPRTNVGPQGX

SEQ ID NO: 262 - protein, 38 aa, Artificial Sequence
  Designed polypeptide
  misc_feature (11)..(11): X = Cit (L-citrulline)
  misc_feature (38)..(38): X = Hyp (L-hydroxyproline)
KCNTATCTVQXLAHQIYQFTDKDKDNVAAPTNVGSNGX

SEQ ID NO: 263 - protein, 38 aa, Artificial Sequence
  Designed polypeptide
  misc_feature (11)..(11): X = Cit (L-citrulline)
GCRFGTCTVQXLAHFLYQFTDKDKDNVAPRTNVGPQGY

SEQ ID NO: 264 - protein, 38 aa, Artificial Sequence
  Designed polypeptide
  misc_feature (11)..(11): X = Cit (L-citrulline)
GCRFGTCTVQXLAHFLYQFTDKDKDNVAPRTNVGSNTY

SEQ ID NO: 265 - protein, 37 aa, Artificial Sequence
  Designed polypeptide
  misc_feature (11)..(11): X = Cit (L-citrulline)
  misc_feature (37)..(37): X = Hyp (L-hydroxyproline)
KCNTATCTVQXLAHQIYQFDKDKDNVAPPTNVGSNGX

SEQ ID NO: 266 - protein, 38 aa, Artificial Sequence
  Designed polypeptide
  misc_feature (11)..(11): X = Cit (L-citrulline)
  misc_feature (38)..(38): X = Hyp (L-hydroxyproline)
KCNTATCTVQXLAEQIYQFTDKDKDNVSPPTNVGSNGX

SEQ ID NO: 267 - protein, 38 aa, Artificial Sequence
  Designed polypeptide
  misc_feature (11)..(11): X = Cit (L-citrulline)
  misc_feature (38)..(38): X = Hyp (L-hydroxyproline)
GCRFGTCTVQXLAHQIYQFTDKDKDNVAPRTNVGPQGX

SEQ ID NO: 268 - protein, 38 aa, Artificial Sequence
  Designed polypeptide
  misc_feature (11)..(11): X = Cit (L-citrulline)
  misc_feature (38)..(38): X = Hyp (L-hydroxyproline)
KCNTATCTVQXLAHQIYQFTDKDKDNVAPPTNVGSNGX

SEQ ID NO: 269 - protein, 38 aa, Artificial Sequence
  Designed polypeptide
  misc_feature (11)..(11): X = Cit (L-citrulline)
GCRTGTCTVQXLAHQIYQFTDKDKDNVAPRTNVGPNGY

SEQ ID NO: 270 - protein, 38 aa, Artificial Sequence
  Designed polypeptide
  misc_feature (11)..(11): X = Cit (L-citrulline)
  misc_feature (38)..(38): X = Hyp (L-hydroxyproline)
GCRFGTCTVQXLAHQIYQFTDKDKDNVAPRTNVGPNGX

SEQ ID NO: 271 - protein, 38 aa, Artificial Sequence
  Designed polypeptide
  misc_feature (11)..(11): X = Cit (L-citrulline)
GCRFGTCTVQXLAHQIYQFTDKDKDNVAPRTNVSPNGY

SEQ ID NO: 272 - protein, 38 aa, Artificial Sequence
  Designed polypeptide
  misc_feature (11)..(11): X = Cit (L-citrulline)
KCNTATCTVQXLAHQIYQFTDKDKDNVAPRTEVGSNGY

SEQ ID NO: 273 - protein, 38 aa, Artificial Sequence
  Designed polypeptide
  misc_feature (11)..(11): X = Cit (L-citrulline)
GCRTGTCTVQXLAHQIYQFTDKDKDNVAPRTNVGPQGY

SEQ ID NO: 274 - protein, 38 aa, Artificial Sequence
  Designed polypeptide
  misc_feature (11)..(11): X = Cit (L-citrulline)
  misc_feature (38)..(38): X = Hyp (L-hydroxyproline)
GCRFGTCTVQXLAHQIYQFTDKDKDNVAPRTKIGPQGX

SEQ ID NO: 275 - protein, 38 aa, Artificial Sequence
  Designed polypeptide
  misc_feature (11)..(11): X = Cit (L-citrulline)
  misc_feature (38)..(38): X = Hyp (L-hydroxyproline)
GCRFGTCTVQXLAHQIYQFTDKDKDNVAPRTKISPNGX

SEQ ID NO: 276 - protein, 38 aa, Artificial Sequence
  Designed polypeptide
  misc_feature (11)..(11): X = Cit (L-citrulline)
  misc_feature (38)..(38): X = Hyp (L-hydroxyproline)
KCNTATCTVQXLAHQIYQATDKDKDNVAPPTNVGSNGX

SEQ ID NO: 277 - protein, 38 aa, Artificial Sequence
  Designed polypeptide
  misc_feature (11)..(11): X = Cit (L-citrulline)
  misc_feature (38)..(38): X = Hyp (L-hydroxyproline)
GCRTGTCTVQXLAHQIYQFTDKDKDNVAPRTKIGPNGX

SEQ ID NO: 278 - protein, 38 aa, Artificial Sequence
  Designed polypeptide
  misc_feature (11)..(11): X = Cit (L-citrulline)
GCRFGTCTVQXLAHQIYQFTDKDKDNVAPRTNVSPQGY

SEQ ID NO: 279 - protein, 38 aa, Artificial Sequence
  Designed polypeptide
  misc_feature (11)..(11): X = Cit (L-citrulline)
GCRFGTCTVQXLAHFLYQFTDKDKDNVAPRTKVGSNGY

SEQ ID NO: 280 - protein, 38 aa, Artificial Sequence
  Designed polypeptide
  misc_feature (11)..(11): X = Cit (L-citrulline)
  misc_feature (38)..(38): X = Hyp (L-hydroxyproline)
GCRTGTCTVQXLAHQIYQFTDKDKDNVAPRTNIGPQGX

SEQ ID NO: 281 - protein, 38 aa, Artificial Sequence
  Designed polypeptide
  misc_feature (11)..(11): X = Cit (L-citrulline)
  misc_feature (38)..(38): X = Hyp (L-hydroxyproline)
GCRTGTCTVQXLAHQIYQFTDKDKDNVAPRSNVGPQGX

SEQ ID NO: 282 - protein, 37 aa, Artificial Sequence
  Designed polypeptide
  misc_feature (11)..(11): X = Cit (L-citrulline)
GCRFGTCTVQXLAHFLYQFTDKDGAIAPRTKIGSQGY

SEQ ID NO: 283 - protein, 38 aa, Artificial Sequence
  Designed polypeptide
  misc_feature (11)..(11): X = Cit (L-citrulline)
  misc_feature (38)..(38): X = Hyp (L-hydroxyproline)
GCRFGTCTVQXLAHQIYQFTDKDKDNVAPRTNVSPQGX

SEQ ID NO: 284 - protein, 38 aa, Artificial Sequence
  Designed polypeptide
  misc_feature (11)..(11): X = Cit (L-citrulline)
  misc_feature (38)..(38): X = Hyp (L-hydroxyproline)
GCRFGTCTVQXLAHQIYQFTDKDKDNVAPRSKIGPQGX

SEQ ID NO: 285 - protein, 38 aa, Artificial Sequence
  Designed polypeptide
  misc_feature (11)..(11): X = Cit (L-citrulline)
GCRTGTCTVQXLAHQIYQFTDKDKDNVAPRSKVGPQGY

SEQ ID NO: 286 - protein, 38 aa, Artificial Sequence
  Designed polypeptide
  misc_feature (11)..(11): X = Cit (L-citrulline)
GCRFGTCTVQXLAHQIYQFTDKDKDNVAPRSNVSPQGY

SEQ ID NO: 287 - protein, 38 aa, Artificial Sequence
  Designed polypeptide
  misc_feature (11)..(11): X = Cit (L-citrulline)
  misc_feature (38)..(38): X = Hyp (L-hydroxyproline)
GCRFGTCTVQXLAHQIYQFTDKDKDNVAPRTKVSPQGX

SEQ ID NO: 288 - protein, 38 aa, Artificial Sequence
  Designed polypeptide
  misc_feature (11)..(11): X = Cit (L-citrulline)
  misc_feature (38)..(38): X = Hyp (L-hydroxyproline)
GCRFGTCTVQXLAHQIYQFTDKDKDNVAPRTKVSPNGX

SEQ ID NO: 289 - protein, 38 aa, Artificial Sequence
  Designed polypeptide
  misc_feature (11)..(11): X = Cit (L-citrulline)
  misc_feature (38)..(38): X = Hyp (L-hydroxyproline)
GCRFGTCTVQXLAHQIYQFTDKDKDNVAPRSNVGPQGX

SEQ ID NO: 290 - protein, 38 aa, Artificial Sequence
  Designed polypeptide
  misc_feature (11)..(11): X = Cit (L-citrulline)
  misc_feature (38)..(38): X = Hyp (L-hydroxyproline)
GCRTGTCTVQXLAHQIYQFTDKDKDNVAPRSKVGPNGX

SEQ ID NO: 291 - protein, 38 aa, Artificial Sequence
  Designed polypeptide
  misc_feature (11)..(11): X = Cit (L-citrulline)
  misc_feature (38)..(38): X = Hyp (L-hydroxyproline)
GCRFGTCTVQXLAHQIYQFTDKDKDNVAPRTNISPQGX

SEQ ID NO: 292 - protein, 38 aa, Artificial Sequence
  Designed polypeptide
  misc_feature (11)..(11): X = Cit (L-citrulline)
  misc_feature (38)..(38): X = Hyp (L-hydroxyproline)
GCRTGTCTVQXLAHQIYQFTDKDKDNVAPRTKVGPQGX

SEQ ID NO: 293 - protein, 38 aa, Artificial Sequence
  Designed polypeptide
  misc_feature (11)..(11): X = Cit (L-citrulline)
  misc_feature (38)..(38): X = Hyp (L-hydroxyproline)
GCRFGTCTVQXLAHQIYQFTDKDKDNVAPRSNVSPQGX

SEQ ID NO: 294 - protein, 38 aa, Artificial Sequence
  Designed polypeptide
  misc_feature (11)..(11): X = Cit (L-citrulline)
  misc_feature (38)..(38): X = Hyp (L-hydroxyproline)
GCRFGTCTVQXLAHQIYQFTDKDKDNVAPRTKISPQGX

SEQ ID NO: 295 - protein, 38 aa, Artificial Sequence
  Designed polypeptide
  misc_feature (11)..(11): X = Cit (L-citrulline)
  misc_feature (38)..(38): X = Hyp (L-hydroxyproline)
GCRIGTCTVQXLAHQIYQFTDKFKDNVAPRSKISPQTX

SEQ ID NO: 296 - protein, 38 aa, Artificial Sequence
  Designed polypeptide
  misc_feature (11)..(11): X = Cit (L-citrulline)
  misc_feature (38)..(38): X = Hyp (L-hydroxyproline)
GCRWGTCTVQXLAHQIYQFTDKDKDNVAPRSKISPQTX

SEQ ID NO: 297 - protein, 38 aa, Artificial Sequence
  Designed polypeptide
  misc_feature (11)..(11): X = Cit (L-citrulline)
  misc_feature (38)..(38): X = Hyp (L-hydroxyproline)
GCRTGTCTVQXLAHQIYQFTDKDKDNVAPRSNIGPNGX

SEQ ID NO: 298 - protein, 38 aa, Artificial Sequence
  Designed polypeptide
  misc_feature (11)..(11): X = Cit (L-citrulline)
GCRTGTCTVQXLAHQIYQFTDKDKDNVAPRTKVGPQGY

SEQ ID NO: 299 - protein, 38 aa, Artificial Sequence
  Designed polypeptide
  misc_feature (11)..(11): X = Cit (L-citrulline)
  misc_feature (38)..(38): X = Hyp (L-hydroxyproline)
GCRTGTCTVQXLAHQIYQFTDKDKDNVAPRSKIGPNGX

SEQ ID NO: 300 - protein, 38 aa, Artificial Sequence
  Designed polypeptide
  misc_feature (11)..(11): X = Cit (L-citrulline)
  misc_feature (38)..(38): X = Hyp (L-hydroxyproline)
GCRFGTCTVQXLAHQIYQFTDKDKDNVAPRSNISPQGX

SEQ ID NO: 301 - protein, 38 aa, Artificial Sequence
  Designed polypeptide
  misc_feature (11)..(11): X = Cit (L-citrulline)
  misc_feature (38)..(38): X = Hyp (L-hydroxyproline)
GCRTGTCTVQXLAHQIYQFTDKDKDNVAPRTKIGPQGX

SEQ ID NO: 302 - protein, 38 aa, Artificial Sequence
  Designed polypeptide
  misc_feature (11)..(11): X = Cit (L-citrulline)
  misc_feature (38)..(38): X = Hyp (L-hydroxyproline)
GCRTGTCTVQXLAHQIYQFTDKDKDNVAPRTNVSPNGX

SEQ ID NO: 303 - protein, 38 aa, Artificial Sequence
  Designed polypeptide
  misc_feature (11)..(11): X = Cit (L-citrulline)
  misc_feature (38)..(38): X = Hyp (L-hydroxyproline)
GCRTGTCTVQXLAHQIYQFTDKDKDNVAPRSNIGPQGX

SEQ ID NO: 304 - protein, 38 aa, Artificial Sequence
  Designed polypeptide
  misc_feature (11)..(11): X = Cit (L-citrulline)
  misc_feature (38)..(38): X = Hyp (L-hydroxyproline)
GCRTGTCTVQXLAHQIYQFTDKDKDNVAPRSNVSPNGX

SEQ ID NO: 305 - protein, 38 aa, Artificial Sequence
  Designed polypeptide
  misc_feature (11)..(11): X = Cit (L-citrulline)
  misc_feature (38)..(38): X = Hyp (L-hydroxyproline)
GCRFGTCTVQXLAHQIYQFTDKDKDNVAPRSKVSPQGX

SEQ ID NO: 306 - protein, 38 aa, Artificial Sequence
  Designed polypeptide
  misc_feature (38)..(38): X = Hyp (L-hydroxyproline)
KCNTSTCTVAWLADQITQFSNKDKAQVSPPTEVGPNSX

SEQ ID NO: 307 - protein, 38 aa, Artificial Sequence
  Designed polypeptide
  misc_feature (38)..(38): X = Hyp (L-hydroxyproline)
RCNASTCTVNWLADQITQFSNKDKAQVSPPTEVGPNSX

SEQ ID NO: 308 - protein, 38 aa, Artificial Sequence
  Designed polypeptide
  misc_feature (38)..(38): X = Hyp (L-hydroxyproline)
KCNTATCTVQWLAHAIYQFTDKDKDNVAPPTNVGSNGX

SEQ ID NO: 309 - protein, 38 aa, Artificial Sequence
  Designed polypeptide
  misc_feature (38)..(38): X = Hyp (L-hydroxyproline)
KCNTATCTVQWLAHQIAQFTDKDKDNVAPPTNVGSNGX

SEQ ID NO: 310 - protein, 38 aa, Artificial Sequence
  Designed polypeptide
  misc_feature (38)..(38): X = Hyp (L-hydroxyproline)
KCNTSTCTVAWLADQITQFSDKDKANVSPPTEVGPNSX

SEQ ID NO: 311 - protein, 38 aa, Artificial Sequence
  Designed polypeptide
GCRFGTCTVQWLANFLYQFTDKDKDNVAPRTNVGPQGY

SEQ ID NO: 312 - protein, 38 aa, Artificial Sequence
  Designed polypeptide
  misc_feature (38)..(38): X = Hyp (L-hydroxyproline)
KCNTATCTVQWLAHQIYQFTDKDKDNVAPRTKVGSNGX

SEQ ID NO: 313 - protein, 38 aa, Artificial Sequence
  Designed polypeptide
  misc_feature (38)..(38): X = Hyp (L-hydroxyproline)
KCNTATCTVQWLAHQIYQFADKDKDNVAPPTNVGSNGX

SEQ ID NO: 314 - protein, 38 aa, Artificial Sequence
  Designed polypeptide
  misc_feature (38)..(38): X = Hyp (L-hydroxyproline)
KCNTATCTVQWLAHQIYQFTDKDKANVAPPTNVGSNGX

SEQ ID NO: 315 - protein, 38 aa, Artificial Sequence
  Designed polypeptide
  misc_feature (38)..(38): X = Hyp (L-hydroxyproline)
KCNTATCTVQWLAHQIYQFTDKDKDNAAPPTNVGSNGX

SEQ ID NO: 316 - protein, 38 aa, Artificial Sequence
  Designed polypeptide
  misc_feature (38)..(38): X = Hyp (L-hydroxyproline)
KCNTATCTVQWLAHQIYQFTDKDKDNVAPATNVGSNGX

SEQ ID NO: 317 - protein, 37 aa, Artificial Sequence
  Designed polypeptide
  misc_feature (37)..(37): X = Hyp (L-hydroxyproline)
KCNTATCTVQWLAHQIYQFTKDKDNVAPPTNVGSNGX

SEQ ID NO: 318 - protein, 37 aa, Artificial Sequence
  Designed polypeptide
  misc_feature (37)..(37): X = Hyp (L-hydroxyproline)
KCNTATCTVQWLAHQIYQFTDKDKDNVPPTNVGSNGX

SEQ ID NO: 319 - protein, 37 aa, Artificial Sequence
  Designed polypeptide
  misc_feature (37)..(37): X = Hyp (L-hydroxyproline)
KCNTATCTVQWLAHQIYQFTDKDKDNVAPTNVGSNGX

SEQ ID NO: 320 - protein, 38 aa, Artificial Sequence
  Designed polypeptide
  misc_feature (38)..(38): X = Hyp (L-hydroxyproline)
KCNTATCTVQWLAHQIYQFTDKAKDNVAPPTNVGSNGX

SEQ ID NO: 321 - protein, 38 aa, Artificial Sequence
  Designed polypeptide
  misc_feature (38)..(38): X = Hyp (L-hydroxyproline)
KCNTATCTVQWLAEQIYQFTDKDKDNVAPPYNEGSNGX

SEQ ID NO: 322 - protein, 38 aa, Artificial Sequence
  Designed polypeptide
  misc_feature (38)..(38): X = Hyp (L-hydroxyproline)
GCRFGTCTVQWLAHQIYQFTDKDKDNVAPRTKVGPQGX

SEQ ID NO: 323 - protein, 38 aa, Artificial Sequence
  Designed polypeptide
  misc_feature (38)..(38): X = Hyp (L-hydroxyproline)
GCRTGTCTVQWLAHQIYQFTDKDKDNVAPRTNVGPQGX

SEQ ID NO: 324 - protein, 38 aa, Artificial Sequence
  Designed polypeptide
  misc_feature (38)..(38): X = Hyp (L-hydroxyproline)
KCNTATCTVQWLAHQIYQFTDKDKDAVAPPTNVGSNGX

SEQ ID NO: 325 - protein, 38 aa, Artificial Sequence
  Designed polypeptide
  misc_feature (38)..(38): X = Hyp (L-hydroxyproline)
KCNTATCTVQWLAHQIYQFTDKDKDNVAAPTNVGSNGX

SEQ ID NO: 326 - protein, 38 aa, Artificial Sequence
  Designed polypeptide
GCRFGTCTVQWLAHFLYQFTDKDKDNVAPRTNVGPQGY

SEQ ID NO: 327 - protein, 38 aa, Artificial Sequence
  Designed polypeptide
GCRFGTCTVQWLAHFLYQFTDKDKDNVAPRTNVGSNTY

SEQ ID NO: 328 - protein, 38 aa, Artificial Sequence
  Designed polypeptide
  misc_feature (38)..(38): X = Hyp (L-hydroxyproline)
KCNTATCTVQWLAHQIYQFTDADKDNVAPPTNVGSNGX

SEQ ID NO: 329 - protein, 37 aa, Artificial Sequence
  Designed polypeptide
  misc_feature (37)..(37): X = Hyp (L-hydroxyproline)
KCNTATCTVQWLAHQIYQFDKDKDNVAPPTNVGSNGX

SEQ ID NO: 330 - protein, 38 aa, Artificial Sequence
  Designed polypeptide
  misc_feature (38)..(38): X = Hyp (L-hydroxyproline)
KCNTATCTVQWLAHQIYQFTDKDKDNVAPPTNVGSNGX

SEQ ID NO: 331 - protein, 38 aa, Artificial Sequence
  Designed polypeptide
  misc_feature (38)..(38): X = Hyp (L-hydroxyproline)
GCRFGTCTVQWLAHQIYQFTDKDKDNVAPRTNIGPNGX

SEQ ID NO: 332 - protein, 38 aa, Artificial Sequence
  Designed polypeptide
GCRTGTCTVQWLAHQIYQFTDKDKDNVAPRTNVGPNGY

SEQ ID NO: 333 - protein, 38 aa, Artificial Sequence
  Designed polypeptide
  misc_feature (38)..(38): X = Hyp (L-hydroxyproline)
KCNAATCTVQWLAEQIYQFTDKDKDNVAPPTNVGSNGX

SEQ ID NO: 334 - protein, 38 aa, Artificial Sequence
  Designed polypeptide
KCNTATCTVQWLAHQIYQFTDKDKDNVAPRTEVGSNGY

SEQ ID NO: 335 - protein, 38 aa, Artificial Sequence
  Designed polypeptide
GCRTGTCTVQWLAHQIYQFTDKDKDNVAPRTNVGPQGY

SEQ ID NO: 336 - protein, 38 aa, Artificial Sequence
  Designed polypeptide
  misc_feature (38)..(38): X = Hyp (L-hydroxyproline)
GCRFGTCTVQWLAHQIYQFTDKDKDNVAPRTKIGPQGX

SEQ ID NO: 337 - protein, 38 aa, Artificial Sequence
  Designed polypeptide
  misc_feature (38)..(38): X = Hyp (L-hydroxyproline)
GCRFGTCTVQWLAHQIYQFTDKDKDNVAPRTKISPNGX

SEQ ID NO: 338 - protein, 38 aa, Artificial Sequence
  Designed polypeptide
  misc_feature (38)..(38): X = Hyp (L-hydroxyproline)
KCNTATCTVQWLAHQIYQATDKDKDNVAPPTNVGSNGX

SEQ ID NO: 339 - protein, 38 aa, Artificial Sequence
  Designed polypeptide
  misc_feature (38)..(38): X = Hyp (L-hydroxyproline)
GCRTGTCTVQWLAHQIYQFTDKDKDNVAPRTKIGPNGX

SEQ ID NO: 340 - protein, 38 aa, Artificial Sequence
  Designed polypeptide
GCRFGTCTVQWLAHQIYQFTDKDKDNVAPRTNVSPQGY

SEQ ID NO: 341 - protein, 38 aa, Artificial Sequence
  Designed polypeptide
  misc_feature (38)..(38): X = Hyp (L-hydroxyproline)
GCRTGTCTVQWLAHQIYQFTDKDKDNVAPRTNIGPQGX

SEQ ID NO: 342 - protein, 38 aa, Artificial Sequence
  Designed polypeptide
  misc_feature (38)..(38): X = Hyp (L-hydroxyproline)
GCRTGTCTVQWLAHQIYQFTDKDKDNVAPRSNVGPQGX

SEQ ID NO: 343 - protein, 38 aa, Artificial Sequence
  Designed polypeptide
  misc_feature (38)..(38): X = Hyp (L-hydroxyproline)
GCRFGTCTVQWLAHQIYQFTDKDKDNVAPRTKIGPNGX

SEQ ID NO: 344 - protein, 38 aa, Artificial Sequence
  Designed polypeptide
GCRTGTCTVQWLAHQIYQFTDKDKDNVAPRSKVGPQGY

SEQ ID NO: 345 - protein, 38 aa, Artificial Sequence
  Designed polypeptide
GCRFGTCTVQWLAHQIYQFTDKDKDNVAPRSNVSPQGY

SEQ ID NO: 346 - protein, 38 aa, Artificial Sequence
  Designed polypeptide
GCRTGTCTVQWLAHQIYQFTDKDKDNVAPRSNVGPQGY

SEQ ID NO: 347 - protein, 38 aa, Artificial Sequence
  Designed polypeptide
  misc_feature (38)..(38): X = Hyp (L-hydroxyproline)
GCRTGTCTVQWLAHQIYQFTDKDKDNVAPRSKVGPNGX

SEQ ID NO: 348 - protein, 38 aa, Artificial Sequence
  Designed polypeptide
GCRTGTCTVQWLAHQIYQFTDKDKDNVAPRTNIGPNGY

SEQ ID NO: 349 - protein, 38 aa, Artificial Sequence
  Designed polypeptide
  misc_feature (38)..(38): X = Hyp (L-hydroxyproline)
GCRTGTCTVQWLAHQIYQFTDKDKDNVAPRTKVGPQGX

SEQ ID NO: 350 - protein, 38 aa, Artificial Sequence
  Designed polypeptide
  misc_feature (38)..(38): X = Hyp (L-hydroxyproline)
GCRFGTCTVQWLAHQIYQFTDKDKDNVAPRTKISPQGX

SEQ ID NO: 351 - protein, 38 aa, Artificial Sequence
  Designed polypeptide
  misc_feature (38)..(38): X = Hyp (L-hydroxyproline)
GCRIGTCTVQWLAHQIYQFTDKFKDNVAPRSKISPQTX

SEQ ID NO: 352 - protein, 38 aa, Artificial Sequence
  Designed polypeptide
  misc_feature (38)..(38): X = Hyp (L-hydroxyproline)
GCRTGTCTVQWLAHQIYQFTDKDKDNVAPRSNIGPNGX

SEQ ID NO: 353 - protein, 38 aa, Artificial Sequence
  Designed polypeptide
  misc_feature (38)..(38): X = Hyp (L-hydroxyproline)
GCRFGTCTVQWLAHQIYQFTDKDKDNVAPRSKVGPQGX

SEQ ID NO: 354 - protein, 38 aa, Artificial Sequence
  Designed polypeptide
GCRTGTCTVQWLAHQIYQFTDKDKDNVAPRTKVGPQGY

SEQ ID NO: 355 - protein, 38 aa, Artificial Sequence
  Designed polypeptide
  misc_feature (38)..(38): X = Hyp (L-hydroxyproline)
GCRTGTCTVQWLAHQIYQFTDKDKDNVAPRSKIGPNGX

SEQ ID NO: 356 - protein, 38 aa, Artificial Sequence
  Designed polypeptide
GCRTGTCTVQWLAHQIYQFTDKDKDNVAPRTNIGPQGY

SEQ ID NO: 357 - protein, 38 aa, Artificial Sequence
  Designed polypeptide
  misc_feature (38)..(38): X = Hyp (L-hydroxyproline)
GCRTGTCTVQWLAHQIYQFTDKDKDNVAPRTKIGPQGX

SEQ ID NO: 358 - protein, 38 aa, Artificial Sequence
  Designed polypeptide
  misc_feature (38)..(38): X = Hyp (L-hydroxyproline)
GCRTGTCTVQWLAHQIYQFTDKDKDNVAPRTNVSPNGX

SEQ ID NO: 359 - protein, 38 aa, Artificial Sequence
  Designed polypeptide
  misc_feature (38)..(38): X = Hyp (L-hydroxyproline)
GCRTGTCTVQWLAHQIYQFTDKDKDNVAPRSNIGPQGX

SEQ ID NO: 360 - protein, 38 aa, Artificial Sequence
  Designed polypeptide
  misc_feature (38)..(38): X = Hyp (L-hydroxyproline)
GCRTGTCTVQWLAHQIYQFTDKDKDNVAPRSNVSPNGX

SEQ ID NO: 361 - protein, 38 aa, Artificial Sequence
  Designed polypeptide
KCNFATCTVQRLAHQIYQFTDKDKDNVAPRTKVGSNGY

SEQ ID NO: 362 - protein, 38 aa, Artificial Sequence
  Designed polypeptide
GCRFGTCTVQRLAHQIYQFTDKDKDNVAPRTNVGPQGY

SEQ ID NO: 363 - protein, 38 aa, Artificial Sequence
  Designed polypeptide
KCNFATCATQRLANFLVQFTDKDKDNVAPRSKIGPQGY

SEQ ID NO: 364 - protein, 38 aa, Artificial Sequence
  Designed polypeptide
GCRFGTCTVQRLAHFLYQFTDKDKDNVAPRTNIGPQGY

SEQ ID NO: 365 - protein, 38 aa, Artificial Sequence
  Designed polypeptide
GCRFGTCTVQRLAHFLYQFTDKDKDNVAPRTKIGPQGY

SEQ ID NO: 366 - protein, 38 aa, Artificial Sequence
  Designed polypeptide
GCRFGTCTVQRLAHQIYQFTDKDKDNVAPRTNISPNGY

SEQ ID NO: 367 - protein, 38 aa, Artificial Sequence
  Designed polypeptide
GCRFGTCTVQRLAHQIYQFTDKDKDNVAPRTKIGPNGY

SEQ ID NO: 368 - protein, 38 aa, Artificial Sequence
  Designed polypeptide
GCRFGTCTVQRLAHQIYQFTDKDKDNVAPRTKVGPQGY

SEQ ID NO: 369 - protein, 38 aa, Artificial Sequence
  Designed polypeptide
GCRFGTCTVQRLAHFLYQFTDKDKDNVAPRTKVGPQGY

SEQ ID NO: 370 - protein, 38 aa, Artificial Sequence
  Designed polypeptide
KCNFATCTVQRLAHQIYQFTDKDKDNVAPRTEVGSNGY

SEQ ID NO: 371 - protein, 38 aa, Artificial Sequence
  Designed polypeptide
GCRFGTCTVQRLAHQIYQFTDKDKDNVAPRTKISPNGY

SEQ ID NO: 372 - protein, 38 aa, Artificial Sequence
  Designed polypeptide
GCRFGTCTVQRLANQIYQFTDKDKDNVAPRTNVGPQGY

SEQ ID NO: 373 - protein, 38 aa, Artificial Sequence
  Designed polypeptide
GCRFGTCTVQRLAHQIYQFTDKDKDNVAPRSNVGPNGY

SEQ ID NO: 374 - protein, 38 aa, Artificial Sequence
  Designed polypeptide
GCRFGTCTVQRLAHQIYQFTDKDKDNVAPRSNVGPQGY

SEQ ID NO: 375 - protein, 38 aa, Artificial Sequence
  Designed polypeptide
GCRFGTCTVQRLAHQIYQFTDKDKDNVAPRSKVGPQGY

SEQ ID NO: 376 - protein, 38 aa, Artificial Sequence
  Designed polypeptide
GCRFGTCTVQRLAHFLYQFTDKDKDNVAPRTKIGSNGY

SEQ ID NO: 377 - protein, 38 aa, Artificial Sequence
  Designed polypeptide
GCRFATCTVQRLAHFLYQFTDKDKDNVAPRTKVGPQGY

SEQ ID NO: 378 - protein, 38 aa, Artificial Sequence; identical to SEQ ID NO: 361
  Designed polypeptide

SEQ ID NO: 379 - protein, 38 aa, Artificial Sequence
  Designed polypeptide
GCRFGTCTVQRLAHQIYQFTDKDKDNVAPRTNIGPQGY

SEQ ID NO: 380 - protein, 38 aa, Artificial Sequence
  Designed polypeptide
GCRFATCTVQRLAHQIYQFTDKDKDNVAPRTKVGPQGY

SEQ ID NO: 381 - protein, 38 aa, Artificial Sequence
  Designed polypeptide
GCRFGTCTVQRLAHQIYQFTDKDKDNVAPRTNIGPNGY

SEQ ID NO: 382 - protein, 38 aa, Artificial Sequence
  Designed polypeptide
GCRFGTCTVQRLAHQIYQFTDKDKDNVAPRSNIGPQGY

SEQ ID NO: 383 - protein, 38 aa, Artificial Sequence
  Designed polypeptide
GCRFGTCTVQRLAHQIYQFTDKDKDNVAPRSNISPNGY

SEQ ID NO: 384 - protein, 38 aa, Artificial Sequence
  Designed polypeptide
GCRFGTCTVQRLAHQIYQFTDKDKDNVAPRSKVSPNGY

SEQ ID NO: 385 - protein, 38 aa, Artificial Sequence
  Designed polypeptide
GCRFGTCTVQRLAHQIYQFTDKDKDNVAPRTKVSPNGY

SEQ ID NO: 386 - protein, 38 aa, Artificial Sequence; identical to SEQ ID NO: 16
  Designed polypeptide

SEQ ID NO: 387 - protein, 38 aa, Artificial Sequence
  Designed polypeptide
GCRFGTCTVQRLAHQIYQFTDKDKDNVAPRSKIGPQGY

SEQ ID NO: 388 - protein, 38 aa, Artificial Sequence; identical to SEQ ID NO: 364
  Designed polypeptide

SEQ ID NO: 389 - protein, 38 aa, Artificial Sequence; identical to SEQ ID NO: 363
  Designed polypeptide

SEQ ID NO: 390 - protein, 38 aa, Artificial Sequence; identical to SEQ ID NO: 365
  Designed polypeptide

SEQ ID NO: 391 - protein, 38 aa, Artificial Sequence
  Designed polypeptide
GCRFGTCTVQRLAHQIYQFTDKDKDNVAPRTKIGPQGY

SEQ ID NO: 392 - protein, 38 aa, Artificial Sequence; identical to SEQ ID NO: 369
  Designed polypeptide